European Patent Specification EP 3 368 567 B1, published October 1, 2025. Title: Humanized anti-DKK2 antibody and uses thereof. Applicant: Yale University Wu, Dianqing Chen, Bo Wu, Hai. The sequence listing filed with the application follows.

SEQUENCE LISTING (5 sequences)

SEQ ID NO: 1 - protein, 452 aa, Artificial Sequence
  Artificially synthesized humanized antibody
QVQVVQSGAEVKKPGASVKVSCKASGYSFTNYWMNWVRQAPGQGLEWMGMIHPSDSETRLNQKFQGRVTLTVDKSSSTAYMELSSLRSEDTAVYYCAREGRLGLRSYAMDYWGQGTLVTVSSASTKGPSVFPLAPSSKSTSGGTAALGCLVKDYFPEPVTVSWNSGALTSGVHTFPAVLQSSGLYSLSSVVTVPSSSLGTQTYICNVNHKPSNTKVDKRVEPKSCDKTHTCPPCPAPELLGGPSVFLFPPKPKDTLMISRTPEVTCVVVDVSHEDPEVKFNWYVDGVEVHNAKTKPREEQYNSTYRVVSVLTVLHQDWLNGKEYKCKVSNKALPAPIEKTISKAKGQPREPQVYTLPPSREEMTKNQVSLTCLVKGFYPSDIAVEWESNGQPENNYKTTPPVLDSDGSFFLYSKLTVDKSRWQQGNVFSCSVMHEALHNHYTQKSLSLSPGK

SEQ ID NO: 2 - protein, 220 aa, Artificial Sequence
  Artificially synthesized humanized antibody
DIVMTQSPDSLAVSLGERATINCKSSQSLLNSSNQKNYLAWYQQKPGQPPKLLVYFASTRESGVPDRFSGSGSGTDFTLTISSLQAEDVAVYFCQQHYITPLTFGGGTKVEIKRTVAAPSVFIFPPSDEQLKSGTASVVCLLNNFYPREAKVQWKVDNALQSGNSQESVTEQDSKDSTYSLSSTLTLSKADYEKHKVYACEVTHQGLSSPVTKSFNRGEC

SEQ ID NO: 3 - protein, 452 aa, Artificial Sequence
  Artificially synthesized humanized antibody
QVQLVQSGSELKKPGASVKVSCKASGYTFTNYWMNWVRQAPGQGLEWMGMIHPSDSETRLNQKFKDRVTITVDKSTSTAYMELSSLRSEDTAVYYCAREGRLGLRSYAMDYWGQGTLVTVSSASTKGPSVFPLAPSSKSTSGGTAALGCLVKDYFPEPVTVSWNSGALTSGVHTFPAVLQSSGLYSLSSVVTVPSSSLGTQTYICNVNHKPSNTKVDKRVEPKSCDKTHTCPPCPAPELLGGPSVFLFPPKPKDTLMISRTPEVTCVVVDVSHEDPEVKFNWYVDGVEVHNAKTKPREEQYNSTYRVVSVLTVLHQDWLNGKEYKCKVSNKALPAPIEKTISKAKGQPREPQVYTLPPSREEMTKNQVSLTCLVKGFYPSDIAVEWESNGQPENNYKTTPPVLDSDGSFFLYSKLTVDKSRWQQGNVFSCSVMHEALHNHYTQKSLSLSPGK

SEQ ID NO: 4 - protein, 259 aa, Homo sapiens
MAALMRSKDSSCCLLLLAAVLMVESSQIGSSRAKLNSIKSSLGGETPGQAANRSAGMYQGLAFGGSKKGKNLGQAYPCSSDKECEVGRYCHSPHQGSSACMVCRRKKKRCHRDGMCCPSTRCNNGICIPVTESILTPHIPALDGTRHRDRNHGHYSNHDLGWQNLGRPHTKMSHIKGHEGDPCLRSSDCIEGFCCARHFWTKICKPVLHQGEVCTKQRKKGSHGLEIFQRCDCAKGLSCKVWKDATYSSKARLHVCQKI

SEQ ID NO: 5 - protein, 15 aa, Artificial Sequence
  Artificially synthesized humanized antibody epitope
KLNSIKSSLGGETPG